European Patent Specification EP 3 541 508 B1, published July 12, 2023. Title: Improved chromatography resin, production and use thereof. Applicant: GE Healthcare. The sequence listing filed with the application follows.

SEQUENCE LISTING (6 sequences)

SEQ ID NO: 1 - protein, 186 aa, Artificial
  Npu DnaE N-terminal intein fragment
MGTALSYETEILTVEYGLLPIGKIVEKRIECTVYSVDNNGNIYTQPVAQWHDRGEQEVFEYCLEDGSLIRATKDHKFMTVDGQMLPIDEIFERELDLMRVDNLPNKLGGGGSGGGGSASMKIEEGKLTNPGVSAWQVNTAYTAGQLVTYNGKTYKCLQPHTSLAGWEPSNVPALWQLQLEHHHHHH

SEQ ID NO: 2 - protein, 121 aa, Artificial
  Npu DnaE N-terminal intein fragment
MGTALSYETEILTVEYGLLPIGKIVEKRIECTVYSVDNNGNIYTQPVAQWHDRGEQEVFEYCLEDGSLIRATKDHKFMTVDGQMLPIDEIFERELDLMRVDNLPNGGGGSGGGGSHHHHHH

SEQ ID NO: 3 - protein, 121 aa, Artificial
  Npu DnaE N-terminal intein fragment
MGTALSYETEILTVEYGLLPIGKIVEKRIESTVYSVDNNGNIYTQPVAQWHDRGEQEVFEYSLEDGSLIRATKDHKFMTVDGQMLPIDEIFERELDLMRVDNLPNGGGGSGGGGSHHHHHH

SEQ ID NO: 4 - protein, 122 aa, Artificial
  Npu DnaE N-terminal intein fragment
MGTALSYETEILTVEYGLLPIGKIVEKRIESTVYSVDNNGNIYTQPVAQWHDRGEQEVFEYSLEDGSLIRATKDHKFMTVDGQMLPIDEIFERELDLMRVDNLPNGGGGSGGGGSHHHHHHC

SEQ ID NO: 5 - protein, 116 aa, Artificial
  Npu DnaE N-terminal intein fragment
MGTALSYETEILTVEYGLLPIGKIVEKRIESTVYSVDNNGNIYTQPVAQWHDRGEQEVFEYSLEDGSLIRATKDHKFMTVDGQMLPIDEIFERELDLMRVDNLPNGGGGSGGGGSC

SEQ ID NO: 6 - protein, 283 aa, Artificial
  Npu DnaE C-terminal intein fragment
MIKIATRKYLGKQNVYGIGVERDHNFALKNGFIASNCFNVSKGEELFTGVVPILVELDGDVNGHKFSVSGEGEGDATYGKLTLKFICTTGKLPVPWPTLVTTLTYGVQCFSRYPDHMKQHDFFKSAMPEGYVQERTIFFKDDGNYKTRAEVKFEGDTLVNRIELKGIDFKEDGNILGHKLEYNYNSHNVYIMADKQKNGIKVNFKIRHNIEDGSVQLADHYQQNTPIGDGPVLLPDNHYLSTQSALSKDPNEKRDHMVLLEFVTAAGITLGMDELLEHHHHHH